European Patent Application EP 4 332 230 A1, published March 6, 2024. Title: Mutant of Corynebacterium glutamicum with enhanced L-lysine productivity and method for preparing L-lysine using the same. Applicant: DAESANG CORPORATION. The sequence listing filed with the application follows.

SEQUENCE LISTING (9 sequences)

SEQ ID NO: 1 - DNA, 352 bp, Artificial Sequence
  Promoter sequence of tkt gene
gattcgttccgttcgtgacgctttgtgaggttttttgacgttgcaccgtattgcttgccgaacatttttcttttcctttcggtttttcgagaattttcacctacaaaagcccacgtcacagctcccagacttaagattgatcacacctttgacacatttgaaccacagttggttataaaatgggttcaacatcactatggttagaggtgttgacgggtcagattaagcaaagactactttcggggtagatcacctttgccaaatttgaaccaattaacctaagtcgtagatctgatcatcggatctaacgaaaacgaaccaaaactttggtcccggtttaacccaggaagga

SEQ ID NO: 2 - DNA, 352 bp, Artificial Sequence
  Mutant promoter sequence of tkt gene
gattcgttccgttcgtgacgctttgtgaggttttttgacgttgcaccgtattgcttgccgaacatttttcttttcctttcggtttttcgagaattttcacctacaaaagcccacgtcacagctcccagacttaagattgatcacacctttgacacatttgaaccacagttggttataaaatgggttcaacatcactatggttagaggtgttgacgggtcagattaagcaaagactactttcggggtagatcacctttgccaaatttgaatgtgctgtcataagtcgtagatctgatcatcggatctaacgaaaacgaaccaaaactttggtcccggtttaacccaggaagga

SEQ ID NO: 3 - DNA, 352 bp, Artificial Sequence
  Mutant promoter sequence of tkt gene
gattcgttccgttcgtgacgctttgtgaggttttttgacgttgcaccgtattgcttgccgaacatttttcttttcctttcggtttttcgagaattttcacctacaaaagcccacgtcacagctcccagacttaagattgatcacacctttgacacatttgaaccacagttggttataaaatgggttcaacatcactatggttagaggtgttgacgggtcagattaagcaaagactactttcggggtagatcacctttgccaaatttgaatgtggtatcataagtcgtagatctgatcatcggatctaacgaaaacgaaccaaaactttggtcccggtttaacccaggaagga

SEQ ID NO: 4 - DNA, 26 bp, Artificial Sequence
  Ptkt-1F
ggaattcccctgggcttcgttagcgc

SEQ ID NO: 5 - DNA, 42 bp, Artificial Sequence
  Ptkt83-1-F2
cctttgccaaatttgaatgtgctgtcataagtcgtagatctg

SEQ ID NO: 6 - DNA, 42 bp, Artificial Sequence
  Ptkt83-1-R1
cagatctacgacttatgacagcacattcaaatttggcaaagg

SEQ ID NO: 7 - DNA, 27 bp, Artificial Sequence
  Ptkt-R2
gggatccctcacgacgagcagccatgg

SEQ ID NO: 8 - DNA, 42 bp, Artificial Sequence
  Ptkt83-7-F2
cctttgccaaatttgaatgtggtatcataagtcgtagatctg

SEQ ID NO: 9 - DNA, 42 bp, Artificial Sequence
  Ptkt83-7-R1
cagatctacgacttatgataccacattcaaatttggcaaagg